European Patent Specification EP 3 402 802 B1, published April 12, 2023. Title: Compositions and Methods for Generating an Immune Response to a Tumor Associated Antigen. Applicant: GeoVax, Inc. The sequence listing filed with the application follows.

SEQUENCE LISTING (38 sequences)

SEQ ID NO: 1 - protein, 20 aa, Homo sapiens
AHGVTSAPDTRPAPGSTAPP

SEQ ID NO: 2 - protein, 20 aa, Homo sapiens
AHGVTSAPDNRPALGSTAPP

SEQ ID NO: 3 - protein, 40 aa, Homo sapiens
AHGVTSAPDTRPAPGSTAPPAHGVTSAPDNRPALGSTAPP

SEQ ID NO: 4 - protein, 100 aa, Homo sapiens
AHGVTSAPDTRPAPGSTAPPAHGVTSAPDTRPAPGSTAPPAHGVTSAPDTRPAPGSTAPPAHGVTSAPDTRPAPGSTAPPAHGVTSAPDNRPALGSTAPP

SEQ ID NO: 5 - DNA, 1428 bp, Homo sapiens
atgacaccgggcacccagtctcctttcttcctgctgctgctcctcacagtgcttacagttgttacgggttctggtcatgcaagctctaccccaggtggagaaaaggagacttcggctacccagagaagttcagtgcccagctctactgagaagaatgctgtgagtatgaccagcagcgtactctccagccacagccccggttcaggctcctccaccactcagggacaggatgtcactctggccccggccacggaaccagcttcaggttcagctgccacctggggacaggatgtcacctcggtcccagtcaccaggccagccctgggctccaccaccccgccagcccacgatgtcacctcagccccggacaacaagccagccccgggctccaccgcccccccagcccacggtgtcacctcggccccggacaccaggccggccccgggctccaccgcccccccagcccatggtgtcacctcggccccggacaacaggcccgccttgggctccaccgcccctccagtccacaatgtcacctcggcctcaggctctgcatcaggctcagcttctactctggtgcacaacggcacctctgccagggctaccacaaccccagccagcaagagcactccattctcaattcccagccaccactctgatactcctaccacccttgccagccatagcaccaagactgatgccagtagcactcaccatagcacggtacctcctctcacctcctccaatcacagcacttctccccagttgtctactggggtctctttctttttcctgtcttttcacatttcaaacctccagtttaattcctctctggaagatcccagcaccgactactaccaagagctgcagagagacatttctgaaatgtttttgcagatttataaacaagggggttttctgggcctctccaatattaagttcaggccaggatctgtggtggtacaattgactctggccttccgagaaggtaccatcaatgtccacgacgtggagacacagttcaatcagtataaaacggaagcagcctctcgatataacctgacgatctcagacgtcagcgtgagtgatgtgccatttcctttctctgcccagtctggggctggggtgccaggctggggcatcgcgctgctggtgctggtctgtgttctggttgcgctggccattgtctatctcattgccttggctgtctgtcagtgccgccgaaagaactacgggcagctggacatctttccagcccgggatacctaccatcctatgagcgagtaccccacctaccacacccatgggcgctatgtgccccctagcagtaccgatcgtagcccctatgagaaggtttctgcaggtaatggtggcagcagcctctcttacacaaacccagcagtggcagccacttctgccaacttgtag

SEQ ID NO: 6 - protein, 475 aa, Homo sapiens
MTPGTQSPFFLLLLLTVLTVVTGSGHASSTPGGEKETSATQRSSVPSSTEKNAVSMTSSVLSSHSPGSGSSTTQGQDVTLAPATEPASGSAATWGQDVTSVPVTRPALGSTTPPAHDVTSAPDNKPAPGSTAPPAHGVTSAPDTRPAPGSTAPPAHGVTSAPDNRPALGSTAPPVHNVTSASGSASGSASTLVHNGTSARATTTPASKSTPFSIPSHHSDTPTTLASHSTKTDASSTHHSTVPPLTSSNHSTSPQLSTGVSFFFLSFHISNLQFNSSLEDPSTDYYQELQRDISEMFLQIYKQGGFLGLSNIKFRPGSVVVQLTLAFREGTINVHDVETQFNQYKTEAASRYNLTISDVSVSDVPFPFSAQSGAGVPGWGIALLVLVCVLVALAIVYLIALAVCQCRRKNYGQLDIFPARDTYHPMSEYPTYHTHGRYVPPSSTDRSPYEKVSAGNGGSSLSYTNPAVAATSANL

SEQ ID NO: 7 - DNA, 1608 bp, Homo sapiens
atgacaccgggcacccagtctcctttcttcctgctgctgctcctcacagtgcttacagttgttacgggttctggtcatgcaagctctaccccaggtggagaaaaggagacttcggctacccagagaagttcagtgcccagctctactgagaagaatgctgtgagtatgaccagcagcgtactctccagccacagccccggttcaggctcctccaccactcagggacaggatgtcactctggccccggccacggaaccagcttcaggttcagctgccacctggggacaggatgtcacctcggtcccagtcaccaggccagccctgggctccaccaccccgccagcccacgatgtcacctcagccccggacaacaagccagccccgggctccaccgcccccccagcccacggtgtcacctcggccccggacaccaggccggccccgggctccaccgcccccccagcccacggtgtcacctcggccccggacaccaggccggccccgggctccaccgcccccccagcccacggtgtcacctcggccccggacaccaggccggccccgggctccaccgcccccccagcccacggtgtcacctcggccccggacaccaggccggccccgggctccaccgcccccccagcccatggtgtcacctcggccccggacaacaggcccgccttgggctccaccgcccctccagtccacaatgtcacctcggcctcaggctctgcatcaggctcagcttctactctggtgcacaacggcacctctgccagggctaccacaaccccagccagcaagagcactccattctcaattcccagccaccactctgatactcctaccacccttgccagccatagcaccaagactgatgccagtagcactcaccatagcacggtacctcctctcacctcctccaatcacagcacttctccccagttgtctactggggtctctttctttttcctgtcttttcacatttcaaacctccagtttaattcctctctggaagatcccagcaccgactactaccaagagctgcagagagacatttctgaaatgtttttgcagatttataaacaagggggttttctgggcctctccaatattaagttcaggccaggatctgtggtggtacaattgactctggccttccgagaaggtaccatcaatgtccacgacgtggagacacagttcaatcagtataaaacggaagcagcctctcgatataacctgacgatctcagacgtcagcgtgagtgatgtgccatttcctttctctgcccagtctggggctggggtgccaggctggggcatcgcgctgctggtgctggtctgtgttctggttgcgctggccattgtctatctcattgccttggctgtctgtcagtgccgccgaaagaactacgggcagctggacatctttccagcccgggatacctaccatcctatgagcgagtaccccacctaccacacccatgggcgctatgtgccccctagcagtaccgatcgtagcccctatgagaaggtttctgcaggtaatggtggcagcagcctctcttacacaaacccagcagtggcagccacttctgccaacttgtag

SEQ ID NO: 8 - protein, 535 aa, Homo sapiens
MTPGTQSPFFLLLLLTVLTVVTGSGHASSTPGGEKETSATQRSSVPSSTEKNAVSMTSSVLSSHSPGSGSSTTQGQDVTLAPATEPASGSAATWGQDVTSVPVTRPALGSTTPPAHDVTSAPDNKPAPGSTAPPAHGVTSAPDTRPAPGSTAPPAHGVTSAPDTRPAPGSTAPPAHGVTSAPDTRPAPGSTAPPAHGVTSAPDTRPAPGSTAPPAHGVTSAPDNRPALGSTAPPVHNVTSASGSASGSASTLVHNGTSARATTTPASKSTPFSIPSHHSDTPTTLASHSTKTDASSTHHSTVPPLTSSNHSTSPQLSTGVSFFFLSFHISNLQFNSSLEDPSTDYYQELQRDISEMFLQIYKQGGFLGLSNIKFRPGSVVVQLTLAFREGTINVHDVETQFNQYKTEAASRYNLTISDVSVSDVPFPFSAQSGAGVPGWGIALLVLVCVLVALAIVYLIALAVCQCRRKNYGQLDIFPARDTYHPMSEYPTYHTHGRYVPPSSTDRSPYEKVSAGNGGSSLSYTNPAVAATSANL

SEQ ID NO: 9 - DNA, 2046 bp, Marburg virus
atgtggactacatgcttctttatcagtctcatcttgatccaagggataaaaactctccctattttggagatagccagtaacgatcaaccccaaaatgtggattcggtatgctccggaactctccagaaaacagaagacgtccatctgatgggatttacactgagcgggcagaaagttgctgattcccctttggaggcatccaagcgatgggctttcaggacaggtgtacctcctaagaatgttgagtatacggaaggggaggaagccaaaacatgctacaatataagtgtaacggatccctctggaaaatccttgctgttagatcctcccaccaacgtccgagactatcctaaatgcaaaactatccatcacattcaaggtcaaaaccctcatgcgcaggggatcgccctccatttgtggggagcatttttcctatatgatcgcattgcctccacaacaatgtaccgaggcaaagtcttcactgaagggaacatagcagccatgattgtcaataagacagtgcacaaaatgattttctcgaggcaaggacaagggtaccgtcacatgaatctgacttctactaataaatattggacaagtagcaacggaacgcaaacaaatgacactggatgctttggtactcttcaagaatacaattctacgaagaaccaaacatgtgctccgtctaaaacacccccaccaccgcccacagcccatccggagatcaaacccacaagcaccccaaccgatgccactagactcaacaccacaaacccaaacagtgatgatgaggatctcacaacatccggctcagggtctggggaacaggaaccctatacgacttctgatgcggtcactaagcaagggctttcatcaacaatgccacccactctctcaccgcaaccaggcacgccacagcaaggaggaaacaacacaaaccactcccaagacgctgcaactgaacttgacaacaccaatacaactgcacaaccgcccatgccctcccacaacaccaccacaatctccaccaacaacacctccaaacacaacctcagcaccctctccgaaccaccacaaaacaccaccaatcccaacacacaaagcatggccactgaaaatgagaaaaccagtgcccccccgaaaacaaccctgcctccaacagaaagtcctaccacagaaaagagcaccaacaatacaaaaagccccaccacaatggaaccaaatacaacaaacggacatttcactagtccctcctccacccccaactcgactactcaacatcttatatatttcaggaggaaacgaagtatcctctggagggaaggcgacatgttcccttttctagatgggttaataaatgctccaattgattttgatccagttccaaatacaaagacaatctttgatgaatcttctagttctggtgcttcagccgaggaagatcaacatgcatcctccaatatcagtttaactttatcttatcttcctcatacaagtgaaaacactgcctactctggagaaaatgaaaatgattgtgatgcagagctaagaatttggagcgttcaggaggacgacctggcagcagggctcagttggataccattttttggccctggaatcgaaggactttataccgctggtttaattaaaaatcaaaacaatttggtctgcaggttgaggcgtctagccaatcaaactgcaaaatctttggaactcttactaagggtcacaaccgaggaaagaacattttctttaatcaatagacatgctattgactttctactcacaaggtggggaggaacatgcaaagtgcttggacccgattgttgcataggaatagaggacttgtccagaaatatttcagaacagattgaccaaatcaagaaggacgaacaaaaagaggggactggttggggtctgggtggtaaatggtggacatccgactggggtgttcttactaacttgggcatcttactactattgtccatagctgtcttgattgctctatcctgtatttgtcgtatctttactaaatatattggatag

SEQ ID NO: 10 - protein, 681 aa, Marburg virus
MWTTCFFISLILIQGIKTLPILEIASNDQPQNVDSVCSGTLQKTEDVHLMGFTLSGQKVADSPLEASKRWAFRTGVPPKNVEYTEGEEAKTCYNISVTDPSGKSLLLDPPTNVRDYPKCKTIHHIQGQNPHAQGIALHLWGAFFLYDRIASTTMYRGKVFTEGNIAAMIVNKTVHKMIFSRQGQGYRHMNLTSTNKYWTSSNGTQTNDTGCFGTLQEYNSTKNQTCAPSKTPPPPPTAHPEIKPTSTPTDATRLNTTNPNSDDEDLTTSGSGSGEQEPYTTSDAVTKQGLSSTMPPTLSPQPGTPQQGGNNTNHSQDAATELDNTNTTAQPPMPSHNTTTISTNNTSKHNLSTLSEPPQNTTNPNTQSMATENEKTSAPPKTTLPPTESPTTEKSTNNTKSPTTMEPNTTNGHFTSPSSTPNSTTQHLIYFRRKRSILWREGDMFPFLDGLINAPIDFDPVPNTKTIFDESSSSGASAEEDQHASSNISLTLSYLPHTSENTAYSGENENDCDAELRIWSVQEDDLAAGLSWIPFFGPGIEGLYTAGLIKNQNNLVCRLRRLANQTAKSLELLLRVTTEERTFSLINRHAIDFLLTRWGGTCKVLGPDCCIGIEDLSRNISEQIDQIKKDEQKEGTGWGLGGKWWTSDWGVLTNLGILLLLSIAVLIALSCICRIFTKYIG

SEQ ID NO: 11 - DNA, 1608 bp, Homo sapiens; identical to SEQ ID NO: 7

SEQ ID NO: 12 - protein, 535 aa, Homo sapiens; identical to SEQ ID NO: 8

SEQ ID NO: 13 - protein, 30 aa, Marburg virus
WWTSDWGVLTNLGILLLLSIAVLIALSCIC

SEQ ID NO: 14 - DNA, 1608 bp, Homo sapiens
atgacaccgggcacccagtctcctttcttcctgctgctgctcctcacagtgcttacagttgttacgggttctggtcatgcaagctctaccccaggtggagaaaaggagacttcggctacccagagaagttcagtgcccagctctactgagaagaatgctgtgagtatgaccagcagcgtactctccagccacagccccggttcaggctcctccaccactcagggacaggatgtcactctggccccggccacggaaccagcttcaggttcagctgccacctggggacaggatgtcacctcggtcccagtcaccaggccagccctgggctccaccaccccgccagcccacgatgtcacctcagccccggacaacaagccagccccgggctccaccgcccccccagcccacggtgtcacctcggccccggacaccaggccggccccgggctccaccgcccccccagcccacggtgtcacctcggccccggacaccaggccggccccgggctccaccgcccccccagcccacggtgtcacctcggccccggacaccaggccggccccgggctccaccgcccccccagcccacggtgtcacctcggccccggacaccaggccggccccgggctccaccgcccccccagcccatggtgtcacctcggccccggacaacaggcccgccttgggctccaccgcccctccagtccacaatgtcacctcggcctcaggctctgcatcaggctcagcttctactctggtgcacaacggcacctctgccagggctaccacaaccccagccagcaagagcactccattctcaattcccagccaccactctgatactcctaccacccttgccagccatagcaccaagactgatgccagtagcactcaccatagcacggtacctcctctcacctcctccaatcacagcacttctccccagttgtctactggggtctctttctttttcctgtcttttcacatttcaaacctccagtttaattcctctctggaagatcccagcaccgactactaccaagagctgcagagagacatttctgaaatgtttttgcagatttataaacaagggggttttctgggcctctccaatattaagttcaggccaggatctgtggtggtacaattgactctggccttccgagaaggtaccatcaatgtccacgacgtggagacacagttcaatcagtataaaacggaagcagcctctcgatataacctgacgatctcagacgtcagcgtgagtgatgtgccatttcctttctctgcccagtctggggctggggtgtggtggacatccgactggggtgttcttactaacttgggcatcttactactattgtccatagctgtcttgattgctctatcctgtatttgtcgccgaaagaactacgggcagctggacatctttccagcccgggatacctaccatcctatgagcgagtaccccacctaccacacccatgggcgctatgtgccccctagcagtaccgatcgtagcccctatgagaaggtttctgcaggtaatggtggcagcagcctctcttacacaaacccagcagtggcagccacttctgccaacttgtag

SEQ ID NO: 15 - protein, 535 aa, Homo sapiens
MTPGTQSPFFLLLLLTVLTVVTGSGHASSTPGGEKETSATQRSSVPSSTEKNAVSMTSSVLSSHSPGSGSSTTQGQDVTLAPATEPASGSAATWGQDVTSVPVTRPALGSTTPPAHDVTSAPDNKPAPGSTAPPAHGVTSAPDTRPAPGSTAPPAHGVTSAPDTRPAPGSTAPPAHGVTSAPDTRPAPGSTAPPAHGVTSAPDTRPAPGSTAPPAHGVTSAPDNRPALGSTAPPVHNVTSASGSASGSASTLVHNGTSARATTTPASKSTPFSIPSHHSDTPTTLASHSTKTDASSTHHSTVPPLTSSNHSTSPQLSTGVSFFFLSFHISNLQFNSSLEDPSTDYYQELQRDISEMFLQIYKQGGFLGLSNIKFRPGSVVVQLTLAFREGTINVHDVETQFNQYKTEAASRYNLTISDVSVSDVPFPFSAQSGAGVWWTSDWGVLTNLGILLLLSIAVLIALSCICRRKNYGQLDIFPARDTYHPMSEYPTYHTHGRYVPPSSTDRSPYEKVSAGNGGSSLSYTNPAVAATSANL

SEQ ID NO: 16 - DNA, 1608 bp, Homo sapiens
atgacacctggaacacaatctccattttttctactactactattgacagtactaacagtagtaacaggatctggacatgcgtctagtacaccaggtggagaaaaagaaacatctgcgactcaaagatcttctgtaccatcttctacagaaaaaaatgcggtatctatgacatctagtgtactatcttctcattctcctggatctggatcttctactacacaaggacaagatgtaacactagcgccagctacagaaccagcttctggatctgctgctacttggggtcaagatgttacttctgttccagtaacaagaccagcgctaggatctacaacaccaccagcgcatgatgtaacaagtgcgccagataataaaccagcgcctggttctactgctccaccagctcatggtgttacttcagcgcctgatacaagacctgcacctggatctacagctcctcctgcacatggtgtaacatctgctccagatacaagaccagctccaggttcaacagcacctccagcgcatggtgttactagtgctccagatacaagacctgcgcctggaagtactgcaccaccagcacatggtgtaactagtgcgcctgatacaagaccagcgccaggatcaactgctcctcctgctcatggtgttacaagtgcacctgataatagacctgcgttgggatctactgcgcctccagttcataatgtaacatcagcgtctggaagtgcgtctggttctgcgtctacattggttcataatggtacatctgcgagagcgacaacaactccagcgtctaaatctacaccattttctattccatctcatcattctgatacaccaacaacattggcgagtcattctacaaaaacagatgcgagttctacacatcattctactgtaccaccactaacatcttctaatcatagtacatctccacaactatctactggtgtatcttttttttttctatcttttcatatttctaatctacagtttaattctagtttggaagatccatctacagattattatcaagaactacaaagagatatttctgaaatgtttctacaaatatataaacaaggaggatttctaggactatctaatattaagtttagaccaggatctgtagtagttcaactaactctagcgtttagagaaggtactattaatgtacatgatgttgaaacacagtttaatcaatataaaacagaagcggcgtctagatataatctaacaatttctgatgtatctgtatctgatgttccatttccattttctgcgcaatctggtgctggtgtatggtggacatctgattggggagtactaactaatctaggaattctactattgctatctattgcggtactaattgcgctatcttgtatatgtagaagaaaaaattatggacaactagatatttttccagcgagagatacttatcatccaatgtctgaatatccaacatatcatacacatggaagatatgtaccaccttcttcaacagatagatctccatatgaaaaagtatctgcgggaaatggtggttcttctctatcttatacaaatccagcggtagcggcgacttctgcgaatctataa

SEQ ID NO: 17 - protein, 535 aa, Homo sapiens; identical to SEQ ID NO: 15

SEQ ID NO: 18 - DNA, 1608 bp, Homo sapiens
atgacacctggaacacaatctccattcttcctactactactattgacagtactaacagtagtaacaggatctggacatgcgtctagtacaccaggtggagagaaggaaacatctgcgactcaaagatcttctgtaccatcttctacagagaagaatgcggtatctatgacatctagtgtactatcttctcattctcctggatctggatcttctactacacaaggacaagatgtaacactagcgccagctacagaaccagcttctggatctgctgctacttggggtcaagatgttacttctgttccagtaacaagaccagcgctaggatctacaacaccaccagcgcatgatgtaacaagtgcgccagataataagccagcgcctggttctactgctccaccagctcatggtgttacttcagcgcctgatacaagacctgcacctggatctacagctcctcctgcacatggtgtaacatctgctccagatacaagaccagctccaggttcaacagcacctccagcgcatggtgttactagtgctccagatacaagacctgcgcctggaagtactgcaccaccagcacatggtgtaactagtgcgcctgatacaagaccagcgccaggatcaactgctcctcctgctcatggtgttacaagtgcacctgataatagacctgcgttgggatctactgcgcctccagttcataatgtaacatcagcgtctggaagtgcgtctggttctgcgtctacattggttcataatggtacatctgcgagagcgacaacaactccagcgtctaagtctacaccattctctattccatctcatcattctgatacaccaacaacattggcgagtcattctacaaagacagatgcgagttctacacatcattctactgtaccaccactaacatcttctaatcatagtacatctccacaactatctactggtgtatctttcttcttcctatcctttcatatttctaatctacagttcaattctagtttggaagatccatctacagattattatcaagaactacaaagagatatttctgaaatgtttctacaaatatataaacaaggaggatttctaggactatctaatattaagtttagaccaggatctgtagtagttcaactaactctagcgtttagagaaggtactattaatgtacatgatgttgaaacacagtttaatcaatataagacagaagcggcgtctagatataatctaacaatttctgatgtatctgtatctgatgttccatttccattttctgcgcaatctggtgctggtgtatggtggacatctgattggggagtactaactaatctaggaattctactattgctatctattgcggtactaattgcgctatcttgtatatgtagaagaaagaattatggacaactagatattttcccagcgagagatacttatcatccaatgtctgaatatccaacatatcatacacatggaagatatgtaccaccttcttcaacagatagatctccatatgagaaggtatctgcgggaaatggtggttcttctctatcttatacaaatccagcggtagcggcgacttctgcgaatctataa

SEQ ID NO: 19 - protein, 535 aa, Homo sapiens; identical to SEQ ID NO: 15

SEQ ID NO: 20 - DNA, 60 bp, Homo sapiens
gctcatggtgttacttcagcgcctgatacaagacctgcacctggatctacagctcctcct

SEQ ID NO: 21 - protein, 20 aa, Homo sapiens
AHGVTSAPDTRPAPGSTAPP

SEQ ID NO: 22 - DNA, 60 bp, Homo sapiens
gcacatggtgtaacatctgctccagatacaagaccagctccaggttcaacagcacctcca

SEQ ID NO: 23 - DNA, 60 bp, Homo sapiens
gcgcatggtgttactagtgctccagatacaagacctgcgcctggaagtactgcaccacca

SEQ ID NO: 24 - DNA, 60 bp, Homo sapiens
gcacatggtgtaactagtgcgcctgatacaagaccagcgccaggatcaactgctcctcct

SEQ ID NO: 25 - DNA, 60 bp, Homo sapiens
gctcatggtgttacttcagcgcctgatacaagacccgcacccggatctaccgctccgcct

SEQ ID NO: 26 - DNA, 60 bp, Homo sapiens
gcacacggcgtcacatctgctcccgacactcgtccagctcctggtagcacagcacctcca

SEQ ID NO: 27 - DNA, 60 bp, Homo sapiens
gcgcatggagtaaccagtgcaccagatacccgacctgcgccgggcagtactgccccaccg

SEQ ID NO: 28 - DNA, 60 bp, Homo sapiens
gcccacggggtgacgagcgccccggacacgcgcccagctccagggtcaacggcgccccct

SEQ ID NO: 29 - DNA, 1633 bp, Homo sapiens
gcgctcccgggatgacacctggaacacaatctccattcttcctactactactattgacagtactaacagtagtaacaggatctggacatgcgtctagtacaccaggtggagagaaggaaacatctgcgactcaaagatcttctgtaccatcttctacagagaagaatgcggtatctatgacatctagtgtactatcttctcattctcctggatctggatcttctactacacaaggacaagatgtaacactagcgccagctacagaaccagcttctggatctgctgctacttggggtcaagatgttacttctgttccagtaacaagaccagcgctaggatctacaacaccaccagcgcatgatgtaacaagtgcgccagataataagccagcgcctggttctactgctccaccagctcatggtgttacttcagcgcctgatacaagacctgcacctggatctacagctcctcctgcacatggtgtaacatctgctccagatacaagaccagctccaggttcaacagcacctccagcgcatggtgttactagtgctccagatacaagacctgcgcctggaagtactgcaccaccagcacatggtgtaactagtgcgcctgatacaagaccagcgccaggatcaactgctcctcctgctcatggtgttacaagtgcacctgataatagacctgcgttgggatctactgcgcctccagttcataatgtaacatcagcgtctggaagtgcgtctggttctgcgtctacattggttcataatggtacatctgcgagagcgacaacaactccagcgtctaagtctacaccattctctattccatctcatcattctgatacaccaacaacattggcgagtcattctacaaagacagatgcgagttctacacatcattctactgtaccaccactaacatcttctaatcatagtacatctccacaactatctactggtgtatctttcttcttcctatcctttcatatttctaatctacagttcaattctagtttggaagatccatctacagattattatcaagaactacaaagagatatttctgaaatgtttctacaaatatataaacaaggaggatttctaggactatctaatattaagtttagaccaggatctgtagtagttcaactaactctagcgtttagagaaggtactattaatgtacatgatgttgaaacacagtttaatcaatataagacagaagcggcgtctagatataatctaacaatttctgatgtatctgtatctgatgttccatttccattctctgcgcaatctggtgctggtgtatggtggacatctgattggggagtactaactaatctaggaattctactattgctatctattgcggtactaattgcgctatcttgtatatgtagaagaaagaattatggacaactagatattttcccagcgagagatacttatcatccaatgtctgaatatccaacatatcatacacatggaagatatgtaccaccttcttcaacagatagatctccatatgagaaggtatctgcgggaaatggtggttcttctctatcttatacaaatccagcggtagcggcgacttctgcgaatctataataagtcgacgcgct

SEQ ID NO: 30 - protein, 535 aa, Homo sapiens; identical to SEQ ID NO: 15

SEQ ID NO: 31 - DNA, 29 bp, Homo sapiens
tatgaatgtagaagcaggagattccagag

SEQ ID NO: 32 - protein, 29 aa, Homo sapiens
TGGTACTGGAATTACAACTATTATCCTCC

SEQ ID NO: 33 - protein, 29 aa, Homo sapiens
CCAAAGAAGGCAGAGATCAACTATACTGG

SEQ ID NO: 34 - DNA, 29 bp, Homo sapiens
acacatagttcctccattgaagacttagc

SEQ ID NO: 35 - DNA, 29 bp, Homo sapiens
taggattggtcatggaaatagaatgcacc

SEQ ID NO: 36 - DNA, 29 bp, Homo sapiens
aaggagacttggaccaaacactgtgacaa

SEQ ID NO: 37 - DNA, 29 bp, Homo sapiens
gcagtttgcctgaaatatgctggagtatt

SEQ ID NO: 38 - DNA, 29 bp, Homo sapiens
cttacctccaaatggttctgacaatgact